European Patent Application EP 4 257 697 A1, published October 11, 2023. Title: Verfahren zur Herstellung von Aromastoffen unter Verwendung einer O-Methyltransferase aus Pleurotus sapidus. Applicant: Justus-Liebig-Universität Gießen. The sequence listing filed with the application follows.

SEQUENCE LISTING (2 sequences)

SEQ ID NO: 1 - protein, 455 aa, Artificial Sequence
  Aminosäuresequenz der O-Methyltransferase aus PSA-Transkriptom
MTTLSPSEGKAQIRALLNLINTSAEQAIAEYDKQECDIPSLTSGEPHPMDDRLPSLELKNTLRILEGACAQLCVTLAPPAHTMLNYSMDVLVPSCISTVIQAGVAPLLAKHPKGLHIDVLSKETGIHPQKLATILRLLILNYCFQEVESNVFANNRLSLTLLPETSVVDILDLKTGEMHRKATLWVYDALVDPDFGPTYDGNKSPLVYALRREGFDGSLYDYLQTQPGAVARFARAMLGFSVSRGLMNLLNVFPWQELAPGSTVCDLGGGNGNTSIEIAKKFPHLKVHLQDLPDTIEEAKVFWKEEYPDAIKDSRVAFTPIDFFKQAPVPDQDIYYISQIVHNWGDEDCITLLKNIRSAMSPKSRLLINDYLASHLDKTSIANQHPSLPRAPYPLSPGFGRGMARTYTGDYTMLVVCNSRERSLEDFIELCSAADLKFVRVWDLAETSVTEFVPA

SEQ ID NO: 2 - protein, 461 aa, Artificial Sequence
  Aminosäuresequenz der O-Methyltransferase in pColdI
MTTLSPSEGKAQIRALLNLINTSAEQAIAEYDKQECDIPSLTSGEPHPMDDRLPSLELKNTLRILEGACAQLCVTLAPPAHTMLNYSMDVLVPSCISTVIQAGVAPLLAKHPKGLHIDVLSKETGIHPQKLATILRLLILNYCFQEVESNVFANNRLSLTLLPETSVVDILDLKTGEMHRKATLWVYDALVDPDFGPTYDGNKSPLVYALRREGFDGSLYDYLQTQPGAVARFARAMLGFSVSRGLMNLLNVFPWQELAPGSTVCDLGGGNGNTSIEIAKKFPHLKVHLQDLPDTIEEAKVFWKEEYPDAIKDSRVAFTPIDFFKQAPVPDQDIYYISQIVHNWGDEDCITLLKNIRSAMSPKSRLLINDYLASHLDKTSIANQHPSLPRAPYPLSPGFGRGMARTYTGDYTMLVVCNSRERSLEDFIELCSAADLKFVRVWDLAETSVTEFVPAHHHHHH